European Patent Application EP 4 310 181 A1, published January 24, 2024. Title: Enzyme Immobilization Carrier and Preparation Method thereof, Immobilized Enzyme and Preparation Method thereof. Applicant: Asymchem Laboratories(Tianjin) Co.,Ltd. The sequence listing filed with the application follows.

SEQUENCE LISTING (5 sequences)

SEQ ID NO: 1 - protein, 459 aa, Artificial Sequence
  Transaminase from Aspergillus fumigatus
MQKQRTCSQWRELDAAHHLHPFTDTASLNQAGARVMTRGEGVYLWDCEGNKIIDGMAGLWCVNVGYGRKDFAEAARRQMEELPFYNTFFGTTHPPVVELSSLLAEVTPAGFDRVFYTNSGSESVDTMIRMVRRYWDVQGKPEKKTLIGRWNGYHGSTIGGASLGGMKYMHEQGDLPIPGMAHIEQPWWYKHGKDMTPDEFGVVAARWLEEKILEIGADKVAAFVGEPIQGAGGVIVPPATYWPEIERICRKYDVLLVADEVICGFGRTGEWFGHQHFGFQPDLFTAAKGLSSGYLPLGAVFVGDRVAEGLIAGGDFNHGFTYSGHPVCAAVAHANVAALRDEGIVQRVKDDIGPYMQKRWRETFSRFEHVDDVRGVGMMLAFTLVKNKAKRELFPDFGEIGTLCEDIFFRNNLIMTAQGDHIVSAPPLVMTRAEVDEMLAVAERCLEEFEQTLKARGLA

SEQ ID NO: 2 - protein, 366 aa, Artificial Sequence
  Leucine Dehydrogenase from Bacillus cereus
MRDVFEMMDRYGHEQVIFCRHPQTGLKAIIALHNTTAGPALGGCRMIPYASTDEALEDVLRLSKGMTYKCSLADVDFGGGKMVIIGDPKKDKSPELFRVIGRFVGGLNGRFYTGTDMGTNPEDFVHAARESKSFAGLPKSYGGKGDTSIPTALGVFHGMRATARFLWGTDQLKGRVVAIQGVGKVGERLLQLLVEVGAYCKIADIDSVRCEQLKEKYGDKVQLVDVNRIHKESCDIFSPCAKGGVVNDDTIDEFRCLAIVGSANNQLVEDRHGALLQKRSICYAPDYLVNAGGLIQVADELEGFHEERVLAKTEAIYDMVLDIFHRAKNENITTCEAADRIVMERLKKLTDIRRILLEDPRNSARR

SEQ ID NO: 3 - protein, 348 aa, Artificial Sequence
  Ketoreductase from Candida macedoniensis AKU4588
MKAIQYTRIGAEPELTEIPKPEPGPGEVLLEVTAAGVCHSDDFIMSLPEEQYTYGLPLTLGHEGAGKVAAVGEGVEGLDIGTNVVVYGPWGCGNCWHCSQGLENYCSRAQELGINPPGLGAPGALAEFMIVDSPRHLVPIGDLDPVKTVPLTDAGLTPYHAIKRSLPKLRGGSYAVVIGTGGLGHVAIQLLRHLSAATVIALDVSADKLELATKVGAHEVVLSDKDAAENVRKITGSQGAALVLDFVGYQPTIDTAMAVAGVGSDVTIVGIGDGQAHAKVGFFQSPYEASVTVPYWGARNELIELIDLAHAGIFDIAVETFSLDNGAEAYRRLAAGTLSGRAVVVPGL

SEQ ID NO: 4 - protein, 603 aa, Artificial Sequence
  Cyclohexanone monooxygenase from Brachymonas petroleovorans
MTTSIDREALRRKYAEERDKRIRPDGNDQYIRLDHVDGWSHDPYMPITPREPKLDHVTFAFIGGGFSGLVTAARLRESGVESVRIIDKAGDFGGVWYWNRYPGAMCDTAAMVYMPLLEETGYMPTEKYAHGPEILEHCQRIGKHYDLYDDALFHTEVTDLVWQEHDQRWRISTNRGDHFTAQFVGMGTGPLHVAQLPGIPGIESFRGKSFHTSRWDYDYTGGDALGAPMDKLADKRVAVIGTGATAVQCVPELAKYCRELYVVQRTPSAVDERGNHPIDEKWFAQIATPGWQKRWLDSFTAIWDGVLTDPSELAIEHEDLVQDGWTALGQRMRAAVGSVPIEQYSPENVQRALEEADDEQMERIRARVDEIVTDPATAAQLKAWFRQMCKRPCFHDDYLPAFNRPNTHLVDTGGKGVERITENGVVVAGVEYEVDCIVYASGFEFLGTGYTDRAGFDPTGRDGVKLSEHWAQGTRTLHGMHTYGFPNLFVLQLMQGAALGSNIPHNFVEAARVVAAIVDHVLSTGTSSVETTKEAEQAWVQLLLDHGRPLGNPECTPGYYNNEGKPAELKDRLNVGYPAGSAAFFRMMDHWLAAGSFDGLTFR

SEQ ID NO: 5 - protein, 340 aa, Artificial Sequence
  Ene Reductase from Saccharomyces cerevisiae
MNTMLFSPYTIRGLTLKNRIVMSPMCMYSCDTKDGAVRTWHKIHYPARAVGQVGLIIVEATGVTPQGRISERDLGIWSDDHIAGLRELVGLVKEHGAAIGIQLAHAGRKSQVPGEIIAPSAVPFDDSSPTPKEMTKADIEETVQAFQNGARRAKEAGFDVIEIHAAHGYLINEFLSPLSNRRQDEYGGSPENRYRFLGEVIDAVREVWDGPLFVRISASDYHPDGLTAKDYVPYAKRMKEQGVDLVDVSSGAIVPARMNVYPGYQVPFAELIRREADIPTGAVGLITSGWQAEEILQNGRADLVFLGRELLRNPYWPYAAARELGAKISAPVQYERGWRF